European Patent Application EP 4 163 296 A1, published April 12, 2023. Title: G-PROTEIN-GATED-K+ CHANNEL-MEDIATED ENHANCEMENTS IN LIGHT SENSITIVITY IN PATIENTS WITH ROD-CONE DYSTROPHY (RCD). Applicant: SPARINGVISION. The sequence listing filed with the application follows.

SEQUENCE LISTING (16 sequences)

SEQ ID NO: 1 - DNA, 1269 bp, Homo sapiens
  source 1..1269: mol_type = unassigned DNA
atggccaagctgacagaatccatgactaacgtcctggagggcgactccatggatcaggacgtcgaaagcccagtggccattcaccagccaaagttgcctaagcaggccagggatgacctgccaagacacatcagccgagatcggaccaaaaggaaaatccagaggtacgtgaggaaagacggaaagtgcaatgttcatcacggcaacgtgagggagacctatcgctacctgaccgatatcttcaccacattagtggacctgaagtggagattcaacctattgatttttgtcatggtttacacagtgacctggctcttttttggaatgatctggtggttgatcgcatacatacggggagacatggaccacatagaggacccctcctggactccttgtgttaccaacctcaacgggttcgtctctgcttttttattctcaatagagacagaaaccaccattggttatggctaccgggtcatcacagataaatgcccagagggaattattcttctcttaatccaatctgtgttggggtccattgtcaatgcattcatggtgggatgcatgtttgtaaaaatctctcaacccaagaagagggcagagaccctggtcttttccacccatgcagtgatctccatgcgggatgggaaactgtgcctgatgttccgggtaggggaccttaggaattcccacattgtggaggcttccatcagagccaagttgatcaaatccaaacagacctcggagggggagttcatcccgttgaaccagacggatatcaacgtagggtattacacgggggatgaccgtctgtttctggtgtcaccgctgatcattagccatgaaattaaccaacagagtcctttctgggagatctccaaagcccagctgcccaaagaggaactggaaattgtggtcatcctagaaggaatggtggaagccacagggatgacatgccaagctcgaagctcctacatcaccagtgagatcctgtggggttaccggttcacacctgtcctgaccctggaggacgggttctacgaagttgactacaacagcttccatgagacctatgagaccagcaccccatcccttagtgccaaagagctggccgagttagccagcagggcagagctgcccctgagttggtctgtatccagcaaactcaaccaacatgcagaactggagactgaagaggaagaaaagaacctcgaagagcaaacagaaagaaatggtgatgtggcaaacctggagaatgaatccaaagtt

SEQ ID NO: 2 - protein, 423 aa, Homo sapiens
MAKLTESMTNVLEGDSMDQDVESPVAIHQPKLPKQARDDLPRHISRDRTKRKIQRYVRKDGKCNVHHGNVRETYRYLTDIFTTLVDLKWRFNLLIFVMVYTVTWLFFGMIWWLIAYIRGDMDHIEDPSWTPCVTNLNGFVSAFLFSIETETTIGYGYRVITDKCPEGIILLLIQSVLGSIVNAFMVGCMFVKISQPKKRAETLVFSTHAVISMRDGKLCLMFRVGDLRNSHIVEASIRAKLIKSKQTSEGEFIPLNQTDINVGYYTGDDRLFLVSPLIISHEINQQSPFWEISKAQLPKEELEIVVILEGMVEATGMTCQARSSYITSEILWGYRFTPVLTLEDGFYEVDYNSFHETYETSTPSLSAKELAELASRAELPLSWSVSSKLNQHAELETEEEEKNLEEQTERNGDVANLENESKV

SEQ ID NO: 3 - DNA, 1275 bp, Mus musculus
  source 1..1275: mol_type = unassigned DNA
atgacaatggccaagttaactgaatccatgactaacgccgccgaaggcgattccatggaccaggatgtggaaagcccagtggccattcaccagccaaagttgcctaagcaggccagggacgacctgccgagacacatcagccgagacaggaccaaaaggaaaatccagaggtacgtgaggaaggatgggaagtgcaacgttcaccacggcaatgtgcgggagacgtaccgatacctgacggacatcttcaccaccctggtggacctgaagtggagattcaacctgttgatctttgtcatggtctacacagtgacgtggcttttctttgggatgatctggtggctgattgcgtacatccggggagatatggaccacatagaggacccctcgtggactccttgtgtcaccaacctcaacgggtttgtctctgcttttttattctccatagagacagaaaccaccatcggttatggctaccgggtcatcacggacaagtgccctgaggggattattctcctcttaatccagtccgtgttggggtccattgtcaacgccttcatggtaggatgtatgtttgtgaaaatatcccaacccaagaagagggcagagaccctggtcttttccacccacgcggtgatctccatgcgggatgggaaactgtgcttgatgttccgggtgggggacttgaggaattctcacattgtggaggcatccatcagagccaagttgatcaagtccaaacagacttcagagggggagtttattcccctcaaccagactgatatcaacgtggggtactacacaggggacgaccggctctttctggtgtcaccattgattattagccatgaaattaaccaacagagtcccttctgggagatctccaaagcgcagctgcctaaagaggaactggagattgtggtcatcctggagggaatggtggaagccacaggaatgacgtgccaagcccgaagctcctacatcaccagtgagatcttgtggggttaccggttcacacctgtcctaacgctggaagacgggttctacgaagttgactacaacagcttccatgagacctatgagaccagcaccccgtcccttagtgccaaagagctagcggagctggctaaccgggcagagctgcctctgagttggtctgtgtccagcaaactgaaccaacatgcagaattggagacagaagaggaagagaagaacccggaagaactgacggagaggaatggtgacgtggcaaacctagagaatgaatccaaagtt

SEQ ID NO: 4 - protein, 425 aa, Mus musculus
MTMAKLTESMTNAAEGDSMDQDVESPVAIHQPKLPKQARDDLPRHISRDRTKRKIQRYVRKDGKCNVHHGNVRETYRYLTDIFTTLVDLKWRFNLLIFVMVYTVTWLFFGMIWWLIAYIRGDMDHIEDPSWTPCVTNLNGFVSAFLFSIETETTIGYGYRVITDKCPEGIILLLIQSVLGSIVNAFMVGCMFVKISQPKKRAETLVFSTHAVISMRDGKLCLMFRVGDLRNSHIVEASIRAKLIKSKQTSEGEFIPLNQTDINVGYYTGDDRLFLVSPLIISHEINQQSPFWEISKAQLPKEELEIVVILEGMVEATGMTCQARSSYITSEILWGYRFTPVLTLEDGFYEVDYNSFHETYETSTPSLSAKELAELANRAELPLSWSVSSKLNQHAELETEEEEKNPEELTERNGDVANLENESKV

SEQ ID NO: 5 - DNA, 1221 bp, Rattus rattus
  source 1..1221: mol_type = unassigned DNA
atggaccaagacgtggaaagcccagtggccattcaccagccaaagttgcctaagcaggccagggatgacctgccaagacacatcagccgagacaggaccaaaaggagaatccagaggtacgtgaggaaggatgggaagtgtaacgtccaccacggcaacgtgcgggagacgtaccgatacctgacggacatcttcaccaccctggtggacctaaagtggagattcaacctattgatctttgtcatggtctacacagtgacgtggcttttctttgggatgatctggtggctaattgcatacatccggggagatatggaccacatagaggacccctcgtggactccctgtgttaccaacctcaacgggtttgtctccgcttttttattctcaatagagacagaaaccaccattggttatggctacagggtcatcacggacaagtgcccagaaggaattattctcctcttaatccagtccgtgttggggtccattgtcaacgccttcatggtaggatgtatgtttgtgaaaatatcccaacccaagaagagggcagagaccctggtcttttccacccatgcggtaatctccatgcgggatgggaaactatgcctgatgttccgggtaggggacttgaggaattcccacattgtggaggcctccatcagagccaagttgatcaagtccaaacagacttcagagggggagttcattcccctcaaccagacggatatcaacgtagggtactacaccggggatgaccgactctttctcgtgtcaccgctgattattagccatgaaattaaccaacagagtcccttctgggagatctccaaagcccagctgcctaaagaggaactggagattgtggtcatcctggagggaatggtggaagccacaggaatgacgtgccaagctcgaagctcctacgtcaccagtgagatcctgtggggttaccggttcacaccagtcctgacactggaggacgggttctatgaagttgactacaacagcttccatgagacccatgagaccagcaccccgtcccttagcgccaaagagctagccgagctggctaaccgggcagagctgcccctgagctggtctgtgtccagcaaactgaaccaacatgcagaactggagacggaagaggaagagaagaacccggaagaactgacagagaggaatggtgatgtggcaaacctagagaatgagtccaaagtg

SEQ ID NO: 6 - protein, 407 aa, Rattus rattus
MDQDVESPVAIHQPKLPKQARDDLPRHISRDRTKRRIQRYVRKDGKCNVHHGNVRETYRYLTDIFTTLVDLKWRFNLLIFVMVYTVTWLFFGMIWWLIAYIRGDMDHIEDPSWTPCVTNLNGFVSAFLFSIETETTIGYGYRVITDKCPEGIILLLIQSVLGSIVNAFMVGCMFVKISQPKKRAETLVFSTHAVISMRDGKLCLMFRVGDLRNSHIVEASIRAKLIKSKQTSEGEFIPLNQTDINVGYYTGDDRLFLVSPLIISHEINQQSPFWEISKAQLPKEELEIVVILEGMVEATGMTCQARSSYVTSEILWGYRFTPVLTLEDGFYEVDYNSFHETHETSTPSLSAKELAELANRAELPLSWSVSSKLNQHAELETEEEEKNPEELTERNGDVANLENESKV

SEQ ID NO: 7 - protein, 7 aa, synthetic construct
LGETTRP

SEQ ID NO: 8 - protein, 732 aa, Adeno-associated virus 9
MAADGYLPDWLEDNLSEGIREWWALKPGAPQPKANQQHQDNARGLVLPGYKYLGPGNGLDKGEPVNAADAAALEHDKAYDQQLKAGDNPYLKYNHADAEFQERLKEDTSFGGNLGRAVFQAKKRLLEPLGLVEEAAKTAPGKKRPVEQSPQEPDSSAGIGKSGAQPAKKRLNFGQTGDTESVPDPQPIGEPPAAPSGVGSLTMASGGGAPVADNNEGADGVGSSSGNWHCDSQWLGDRVITTSTRTWALPTYNNHLYKQISNSTSGGSSNDNAYGYSTPWGYFDFNRFHCHFSPRDWQRLINNNWGFRPKRLNFKLFNIQVKEVTDNNGVKTIANNLTSTVQVFTDSDYQLPYVLGSAHEGCLPPFPADVFMIPQYGYLTLNDGSQAVGRSSFYCLEYFPSQMLRTGNNFQFSYEFENVPFHSSYAHSQSLDRLMNPLIDQYLYYLSKTINGSGQNQQTLKFSVAGPSNMAVQGRNYIPGPSYRQQRVSTTVTQNNNSEFAWPGASSWALNGRNSLMNPGPAMASHKEGEDRFFPLSGSLIFGKQGTGRDNVDADKVMITNEEEIKTTNPVATESYGQVATNHQSAQQAQTGWVQNQGILPGMVWQDRDVYLQGPIWAKIPHTDGNFHPSPLMGGFGMKHPPPQILIKNTPVPADPPTAFNKDKLNSFITQYSTGQVSVEIEWELQKENSKRWNPEIQYTSNYYKSNNVEFAVNTEGVYSEPRPIGTRYLTR

SEQ ID NO: 9 - protein, 735 aa, Adeno-associated virus 2 [sequence omitted]

SEQ ID NO: 10 - protein, 10 aa, synthetic construct
AALGETTRPA

SEQ ID NO: 11 - protein, 10 aa, synthetic construct
LALGETTRPA

SEQ ID NO: 12 - protein, 9 aa, synthetic construct
GLGETTRPA

SEQ ID NO: 13 - DNA, 1724 bp, synthetic construct
  source 1..1724: mol_type = other DNA
ggaggctgaggggtggggaaagggcatgggtgtttcatgaggacagagcttccgtttcatgcaatgaaaagagtttggagacggatggtggtgactggactatacacttacacacggtagcgatggtacactttgtattatgtatattttaccacgatctttttaaagtgtcaaaggcaaatggccaaatggttccttgtcctatagctgtagcagccatcggctgttagtgacaaagcccctgagtcaagatgacagcagcccccataactcctaatcggctctcccgcgtggagtcatttaggagtagtcgcattagagacaagtccaacatctaatcttccaccctggccagggccccagctggcagcgagggtgggagactccgggcagagcagagggcgctgacattggggcccggcctggcttgggtccctctggcctttccccaggggccctctttccttggggctttcttgggccgccactgctcccgctcctctccccccatcccaccccctcaccccctcgttcttcatatccttctctagtgctccctccactttcatccacccttctgcaagagtgtgggaccacaaatgagttttcacctggcctggggacacacgtgcccccacaggtgctgagtgactttctaggacagtaatctgctttaggctaaaatgggacttgatcttctgttagccctaatcatcaattagcagagccggtgaaggtgcagaacctaccgcctttccaggcctcctcccacctctgccacctccactctccttcctgggatgtgggggctggcacacgtgtggcccagggcattggtgggattgcactgagctgggtcattagcgtaatcctggacaagggcagacagggcgagcggagggccagctccggggctcaggcaaggctgggggcttcccccagacaccccactcctcctctgctggacccccacttcatagggcacttcgtgttctcaaagggcttccaaatagcatggtggccttggatgcccagggaagcctcagagttgcttatctccctctagacagaaggggaatctcggtcaagagggagaggtcgccctgttcaaggccacccagccagctcatggcggtaatgggacaaggctggccagccatcccaccctcagaagggacccggtggggcaggtgatctcagaggaggctcacttctgggtctcacattcttggatccggttccaggcctcggccctaaatagtctccctgggctttcaagagaaccacatgagaaaggaggattcgggctctgagcagtttcaccacccaccccccagtctgcaaatcctgacccgtgggtccacctgccccaaaggcggacgcaggacagtagaagggaacagagaacacataaacacagagagggccacagcggctcccacagtcaccgccaccttcctggcggggatgggtggggcgtctgagtttggttcccagcaaatccctctgagccgcccttgcgggctcgcctcaggagcaggggagcaagaggtgggaggaggaggtctaagtcccaggcccaattaagagatcaggtagtgtagggtttgggagcttttaaggtgaagaggcccgggctgatcccacaggccagtataaagcgccgtgaccctcaggtgatgcgccagggccggctgccgtcggggacagggctttccatagcc

SEQ ID NO: 14 - DNA, 234 bp, synthetic construct
  source 1..234: mol_type = other DNA
ccagcaaatccctctgagccgcccccgggggctcgcctcaggagcaaggaagcaaggggtgggaggaggaggtctaagtcccaggcccaattaagagatcagatggtgtaggatttgggagcttttaaggtgaagaggcccgggctgatcccactggccggtataaagcaccgtgaccctcaggtgacgcaccagggccggctgccgtcggggacagggctttccatagcccag

SEQ ID NO: 15 - DNA, 1958 bp, synthetic construct
  source 1..1958: mol_type = other DNA
cctacagcagccagggtgagattatgaggctgagctgagaatatcaagactgtaccgagtagggggccttggcaagtgtggagagcccggcagctggggcagagggcggagtacggtgtgcgtttacggacctcttcaaacgaggtaggaaggtcagaagtcaaaaagggaacaaatgatgtttaaccacacaaaaatgaaaatccaatggttggatatccattccaaatacacaaaggcaacggataagtgatccgggccaggcacagaaggccatgcacccgtaggattgcactcagagctcccaaatgcataggaatagaagggtgggtgcaggaggctgaggggtggggaaagggcatgggtgtttcatgaggacagagcttccgtttcatgcaatgaaaagagtttggagacggatggtggtgactggactatacacttacacacggtagcgatggtacactttgtattatgtatattttaccacgatctttttaaagtgtcaaaggcaaatggccaaatggttccttgtcctatagctgtagcagccatcggctgttagtgacaaagcccctgagtcaagatgacagcagcccccataactcctaatcggctctcccgcgtggagtcatttaggagtagtcgcattagagacaagtccaacatctaatcttccaccctggccagggccccagctggcagcgagggtgggagactccgggcagagcagagggcgctgacattggggcccggcctggcttgggtccctctggcctttccccaggggccctctttccttggggctttcttgggccgccactgctcccgctcctctccccccatcccaccccctcaccccctcgttcttcatatccttctctagtgctccctccactttcatccacccttctgcaagagtgtgggaccacaaatgagttttcacctggcctggggacacacgtgcccccacaggtgctgagtgactttctaggacagtaatctgctttaggctaaaatgggacttgatcttctgttagccctaatcatcaattagcagagccggtgaaggtgcagaacctaccgcctttccaggcctcctcccacctctgccacctccactctccttcctgggatgtgggggctggcacacgtgtggcccagggcattggtgggattgcactgagctgggtcattagcgtaatcctggacaagggcagacagggcgagcggagggccagctccggggctcaggcaaggctgggggcttcccccagacaccccactcctcctctgctggacccccacttcatagggcacttcgtgttctcaaagggcttccaaatagcatggtggccttggatgcccagggaagcctcagagttgcttatctccctctagacagaaggggaatctcggtcaagagggagaggtcgccctgttcaaggccacccagccagctcatggcggtaatgggacaaggctggccagccatcccaccctcagaagggacccggtggggcaggtgatctcagaggaggctcacttctgggtctcacattcttccagcaaatccctctgagccgcccccgggggctcgcctcaggagcaaggaagcaaggggtgggaggaggaggtctaagtcccaggcccaattaagagatcagatggtgtaggatttgggagcttttaaggtgaagaggcccgggctgatcccactggccggtataaagcaccgtgaccctcaggtgacgcaccagggccggctgccgtcggggacagggctttccatagcccaggtaagtatcaaggttacaagacaggtttaaggagaccaatagaaactgggcttgtcgagacagagaagactcttgcgtttctgataggcacctattggtcttactgacatccactttgcctttctctccacaggcccagagaggagacaggccgccacc

SEQ ID NO: 16 - protein, 410 aa, Homo sapiens
MVLKAEHTRSPSATLPSNVPSCRSLSSSEDGPSGPSSLADGGLAHNLQDSVRHRILYLSEQLRVEKASRDGNTVSYLKLVSKADRHQVPHIQQAFEKVNQRASATIAQIEHRLHQCHQQLQELEEGCRPEGLLLMAESDPANCEPPSEKALLSEPPEPGGEDGPVNLPHASRPFILESRFQSLQQGTCLETEDVAQQQNLLLQKVKAELEEAKRFHISLQESYHSLKERSLTDLQLLLESLQEEKCRQALMEEQVNGRLQGQLNEIYNLKHNLACSEERMAYLSYERAKEIWEITETFKSRISKLEMLQQVTQLEAAEHLQSRPPQMLFKFLSPRLSLATVLLVFVSTLCACPSSLISSRLCTCTMLMLIGLGVLAWQRWRAIPATDWQEWVPSRCRLYSKDSGPPADGP